European Patent Application EP 4 474 477 A1, published December 11, 2024. Title: GENETICALLY ENGINEERED STRAINS WITH REDUCED BYPRODUCT FORMATION. Applicant: DSM IP Assets B.V. Application EP. The sequence listing filed with the application follows.

SEQUENCE LISTING (36 sequences)

SEQ ID NO: 1 - DNA, 2292 bp, Escherichia coli
  source 1..2292: mol_type = genomic DNA
ttgtcagaactactctctttcgccctttttctcgcctctgtgctgatttacgcatggaaagcgggacgtaacacctggtggtttgcagccacgttaacggtgctggggctatttgtcgttttaaatatcaccctgtttgccagcgactattttactggcgatggtattaacgacgcggttctctataccttaaccaacagcctgaccggtgctggcgtcagcaaatacattttgccgggtatcggcattgtgctggggctgacagcggtgttcggtgcgctgggctggatcctgcgccgtcgtcgccatcatccgcaccattttggttacagcctgctggcgctcttactggcgctgggttcggtggacgccagcccggcatttcgtcagataacggaactggtgaaatcccagtcacgcgacggcgacccggactttgcggcttattataaagagccgtcgaaaactatccctgacccgaaactcaacctggtttatatctacggcgaaagtctcgagcggacctattttgataacgaggctttcccggatctcacgcctgaactgggcgcgttgaaaaatgaaggcctggatttcagccacacgcagcagctgccgggaacagattacacgattgcgggcatggtggcttctcagtgcggcataccgctgtttgccccctttgaaggcaacgcctccgcctctgtctccagcttcttcccgcagaacatctgtctgggagatatcctgaaaaactcgggttatcagaactatttcgtgcagggcgcgaatctgcgttttgccggtaaagatgtgttcctgaagtcgcatggcttcgaccacttatacggctcagaagagctgaaaagcgtggtagccgacccgcactatcgcaacgactggggattctacgacgataccgttctcgatgaagcgtggaaaaagtttgaagagctttcccgctcaggtcagcgattctcactgtttaccctgacagtcgatacccatcacccggatggttttatctctcgtacctgtaaccgcaaaaaatatgattttgacggtaaaccgaatcagtcattcagcgcggtaagttgcagccaggagaacatcgcgacgtttatcaacaaaatcaaagcgtcaccgtggtttaaagataccgtcatcgtcgtctcttctgaccatttagcgatgaacaacacggcgtggaaatacctcaataagcaggatcgcaataacctgttttttgtcattcgtggcgacaagccgcagcaagagacgctggcagtgaagcgtaacacgatggataacggcgcgacggtgctggacattctcggtggcgataactatctcggacttggtcgtagcagtttatccgggcagtcgatgtcggaaatcttcctcaatatcaaagagaaaacattggcgtggaagccagatatcatccgcctgtggaaattccctaaagagatgaaagagttcaccatcgaccagcagaaaaacatgattgccttctcgggtagccatttccgtttgccgctgctgttgcgggtttcagacaaacgcgtggaaccgctgccggaaagcgaatactcagcaccgctgcgtttccagctggccgatttcgctccacgcgacaatttcgtctgggttgaccgttgctacaagatggcacaactctgggctccggaactggcactttccaccgactggtgtgtctcgcaagggcagcttggcggtcagcaaattgttcagcatgttgacaaaacaacatggcagggcaaaacggcatttaaagatacggtcatcgacatggcgcgttacaaaggcaatgtcgatacgctgaagattgttgataacgatattcgctacaaagccgacagtttcatctttaacgtcgccggtgcgccagaagaggtgaaacagtttagcgggatttcccgtccggagtcgtggggccgctggtccaacgcgcagctgggcgatgaagtaaaaatcgagtacaagcatccgctgccgaagaaatttgacctggtgattaccgccaaagcatacggcaataacgccagccgtcctattccggtacgcgtaggcaatgaagaacaaactcttgtgctgggcaatgaagtgaccaccaccacactgcatttcgataacccaaccgatgccgacacactggtaattgtgccgccggaacctgtctcaaccaacgaagggaatatcctcggacactcgccgcgtaagctcgggatcggcatggtggaaattaaagtggtagaacgtgaagggtaa

SEQ ID NO: 2 - DNA, 1584 bp, Escherichia coli
  source 1..1584: mol_type = genomic DNA
atgaatttaaccctcaaagaatcgcttgttacccgtagccgggtatttagcccgtggactgcgttctactttttacagtcgctattaattaacctcggcttaggttaccccttcagtttgctctacaccgctgcgtttacggctattttgcttttgctatggcgaacattgcctcgcgtacaaaaagttctggtcggtgtcagttcgctggtggcggcttgttatttcccttttgctcaggcctacggcgcgcctaatttcaatacattgctggcattgcactccaccaatatggaagagtcgaccgaaatcctgacgatttttccgtggtacagctacctggtcggcttatttatttttgcgctcggcgtaatagcaatcaggcgaaaaaaagagaatgaaaaagcgcgctggaataccttcgacagcctgtgtctggtattcagtgtggcgacattttttgttgctcccgtgcaaaacctggcctggggtggcgtatttaaactgaaagatactggctatccggtatttcgttttgctaaggatgtcatcgtcaataataacgaggtgattgaagagcaagaacggatggcaaaactttccggaatgaaagatacctggacggtcactgccgttaagccgaagtatcagacctatgtggtggtgatcggtgaaagcgcgcgtcgcgatgccctcggtgcctttggcggtcactgggacaataccccgtttgccagcagcgttaacggtttgatatttgctgactacattgccgccagtggctccacgcagaaatcgcttggcttaacgctcaatcgcgttgtcgatggcaaaccacagtttcaggataactttgtcaccctggcaaatcgcgcgggcttccagacctggtggttttccaaccagggtcaaatcggcgaatacgataccgctatcgccagcatcgccaaacgagcagatgaagtgtacttcctgaaagaaggtaattttgaagcagataaaaacaccaaagacgaagcgttactggatatgaccgctcaagtgctggcgcaagagcactcgcaaccgcagctgattgttctacatctgatgggctcacatccgcaggcctgcgacaggacacaaggaaaatacgaaacctttgtgcaatcgaaagaaacgtcgtgctatctctataccatgacgcaaacggacgatttactgcgcaagctgtacgatcagttacgcaacagcggcagcagcttctcgctggtttacttttctgaccacggtctggcctttaaagagcgcggtaaagacgtgcaataccttgcccatgatgataaatatcagcaaaatttccaggtgccttttatggtcatttccagcgacgataaagcgcatcgtgtgattaaagcccgccgctcagccaatgacttcttaggctttttctcccagtggacggggattaaagcgaaggaaattaacatcaaatacccgtttatatctgagaagaaagccgggccgatatacatcaccaacttccagttacagaaggtggattacaaccatctcggaaccgatattttcgacccgaaaccttaa

SEQ ID NO: 3 - protein, 763 aa, Escherichia coli
MSELLSFALFLASVLIYAWKAGRNTWWFAATLTVLGLFVVLNITLFASDYFTGDGINDAVLYTLTNSLTGAGVSKYILPGIGIVLGLTAVFGALGWILRRRRHHPHHFGYSLLALLLALGSVDASPAFRQITELVKSQSRDGDPDFAAYYKEPSKTIPDPKLNLVYIYGESLERTYFDNEAFPDLTPELGALKNEGLDFSHTQQLPGTDYTIAGMVASQCGIPLFAPFEGNASASVSSFFPQNICLGDILKNSGYQNYFVQGANLRFAGKDVFLKSHGFDHLYGSEELKSVVADPHYRNDWGFYDDTVLDEAWKKFEELSRSGQRFSLFTLTVDTHHPDGFISRTCNRKKYDFDGKPNQSFSAVSCSQENIATFINKIKASPWFKDTVIVVSSDHLAMNNTAWKYLNKQDRNNLFFVIRGDKPQQETLAVKRNTMDNGATVLDILGGDNYLGLGRSSLSGQSMSEIFLNIKEKTLAWKPDIIRLWKFPKEMKEFTIDQQKNMIAFSGSHFRLPLLLRVSDKRVEPLPESEYSAPLRFQLADFAPRDNFVWVDRCYKMAQLWAPELALSTDWCVSQGQLGGQQIVQHVDKTTWQGKTAFKDTVIDMARYKGNVDTLKIVDNDIRYKADSFIFNVAGAPEEVKQFSGISRPESWGRWSNAQLGDEVKIEYKHPLPKKFDLVITAKAYGNNASRPIPVRVGNEEQTLVLGNEVTTTTLHFDNPTDADTLVIVPPEPVSTNEGNILGHSPRKLGIGMVEIKVVEREG

SEQ ID NO: 4 - protein, 527 aa, Escherichia coli
MNLTLKESLVTRSRVFSPWTAFYFLQSLLINLGLGYPFSLLYTAAFTAILLLLWRTLPRVQKVLVGVSSLVAACYFPFAQAYGAPNFNTLLALHSTNMEESTEILTIFPWYSYLVGLFIFALGVIAIRRKKENEKARWNTFDSLCLVFSVATFFVAPVQNLAWGGVFKLKDTGYPVFRFAKDVIVNNNEVIEEQERMAKLSGMKDTWTVTAVKPKYQTYVVVIGESARRDALGAFGGHWDNTPFASSVNGLIFADYIAASGSTQKSLGLTLNRVVDGKPQFQDNFVTLANRAGFQTWWFSNQGQIGEYDTAIASIAKRADEVYFLKEGNFEADKNTKDEALLDMTAQVLAQEHSQPQLIVLHLMGSHPQACDRTQGKYETFVQSKETSCYLYTMTQTDDLLRKLYDQLRNSGSSFSLVYFSDHGLAFKERGKDVQYLAHDDKYQQNFQVPFMVISSDDKAHRVIKARRSANDFLGFFSQWTGIKAKEINIKYPFISEKKAGPIYITNFQLQKVDYNHLGTDIFDPKP

SEQ ID NO: 5 - protein, 394 aa, Rosenbergiella nectarea
MQSFTPPAPKGGNPVFMMFMLVTFFVSIAGALQAPTLSLYLSQELAAKPFMVGLFFTINAVTGIIISFILAKRSDRKGDRRRLLMFCCAMAIANALMFAFVRQYVVLITLGLILSALTSVVMPQLFALAREYADRTGREVVMFSSVMRTQMSLAWVIGPPISFALALNYGFITLYLVAAALFLLSLILIKTTLPSVPRLYPAEDLAKSAASGWKRTDVRFLFAASVLMWVCNLMYIIDMPLYISKSLGMPESFAGVLMGTAAGLEIPVMLLAGYLAKRVGKRPLVIVAAVCGLAFYPAMLVFHQQTGLLIIQLLNAVFIGIVAGLVMLWFQDLMPGKAGAATTLFTNSVSTGMIFAGLCQGLLSDLLGHQAIYVLATVLMVIALLLLLRVKEQA

SEQ ID NO: 6 - protein, 332 aa, Neisseria meningitidis
MQPLVSVLICAYNVEKYFAQSLAAVVNQTWRNLEILIVDDGSTDGTLAIAKDFQKRDSRIKILAQAQNSGLIPSLNIGLDELAKSGMGEYIARTDADDIAAPDWIEKIVGEMEKDRSIIAMGAWLEVLSEEKDGNRLARHHRHGKIWKKPTRPEDIADFFPFGNPIHNNTMIMRRSVIDGGLRYNTERDWAEDYQFWYDVSKLGRLAYYPEALVKYRLHANQVSSKYSIRQHEIAQGIQKTARNDFLQSMGFKTRFDSLEYRQIKAVAYELLEKHLPEEDFERARRFLYQCFKRTDTLPAGAWLDFAADGRMRRLFTLRQYFGILHRLLKNR

SEQ ID NO: 7 - protein, 439 aa, Helicobacter pylori
MISVYIISLKESQRRLDTEKLVLESNEKFKGRCVFQIFDAISPKHEDFEKFVQELYDSSSLLKSDWFHSDYCYQELLPQEFGCYLSHYLLWKECVKLNQPVVILEDDVALESNFMQALEDCLKSPFDFVRLYGHYWGGHKTNLCALPVYTETEEAEASIEKTPIENYEVTSPPPPNPTRDTQQDFITETQQDPKELSEPCKIAPQKISFNQVVFKKIKRKLNRFIGSILARTEVYKNIVAKYDDLTTKYDDLTTKYDDLTTKYDDLTTKYDDLNKNIAEKYDELMGKYESLLAKEVNIKETFWESRADSEKEALFLDHFYLTSVYVATTAGYYLTPKGAKTFIEATERFKIIEPVDMFINNPTYHDIANFTYVPCPVSLNKHAFNSTIQNAKKPDISLKPPKKSYFDNLFYHKFNARKCLKAFNKYSKQYAPLKTPKEV

SEQ ID NO: 8 - protein, 273 aa, Helicobacter pylori
MRVFAISLNQKVCDTFGLVFRDTTTLLNSINATHHQAQIFDAIYSKTFEGGLHPLVKKHLHPYFITQNIKDMGITTNLISEVSKFYYALKYHAKFMSLGELGCYASHYSLWEKCIELNEAICILEDDITLKEDFKEGLDFLEKHIQELGYIRLMHLLYDASVKSEPLSHKNHEIQERVGIIKAYSEGVGTQGYVITPKIAKVFLKCSRKWVVPVDTIMDATFIHGVKNLVLQPFVIADDEQISTIARKEEPYSPKIALMRELHFKYLKYWQFV

SEQ ID NO: 9 - protein, 417 aa, Escherichia coli [sequence omitted]

SEQ ID NO: 10 - DNA, 203 bp, Synthetic construct
  source 1..203: mol_type = other DNA
tgcgtcgccattctgtcgcaacacgccagaatgcggcggcgatcactaactcaacaaatcaggcgatgtaaccgctttcaatctgtgagtgatttcacagtatcttaacaatgtgatagctatgattgcaccgtgcctacaagcatcgtggaggtccgtgactttcacgcatacaacaaacattaaccaagagaaaaacagct

SEQ ID NO: 11 - DNA, 203 bp, Synthetic construct
  source 1..203: mol_type = other DNA
tgcgtcgccattctgtcgcaacacgccagaatgcggcggcgatcactaactcaacaaatcaggcgatgtaaccgctttcaatctgtgagtgatttcacagtatcttaacaatgtgatagctatgattgcaccgtgcctacaagcatcgtggaggtccgtgactttcacgcatacaacaaacattaaccaactgagaaacagct

SEQ ID NO: 12 - DNA, 203 bp, Synthetic construct
  source 1..203: mol_type = other DNA
tgcgtcgccattctgtcgcaacacgccagaatgcggcggcgatcactaactcaacaaatcaggcgatgtaaccgctttcaatctgtgagtgatttcacagtatcttaacaatgtgatagctatgattgcaccgtgcctacaagcatcgtggaggtccgtgactttcacgcatacaacaaacattaacaaaaaccggagatacc

SEQ ID NO: 13 - DNA, 141 bp, Synthetic construct
  source 1..141: mol_type = other DNA
tgtgagttagctcactcattaggcaccccaggctttacactttatgcttccggctcgtatgttgtgtggaatgcctacaagcatcgtggaggtccgtgactttcacgcatacaacaaacattaaccaaggaggaaacagct

SEQ ID NO: 14 - DNA, 203 bp, Synthetic construct
  source 1..203: mol_type = other DNA
tgcgtcgccattctgtcgcaacacgccagaatgcggcggcgatcactaactcaacaaatcaggcgatgtaaccgctttcaatctgtgagtgatttcacagtatcttaacaatgtgatagctatgattgcaccgtgcctacaagcatcgtggaggtccgtgactttcacgcatacaacaaacattaaccaaaggaaaaacagct

SEQ ID NO: 15 - DNA, 203 bp, Synthetic construct
  source 1..203: mol_type = other DNA
tgcgtcgccattctgtcgcaacacgccagaatgcggcggcgatcactaactcaacaaatcaggcgatgtaaccgctttcaatctgtgagtgatttcacagtatcttaacaatgtgatagctatgattgcaccgtgcctacaagcatcgtggaggtccgtgactttcacgcatacaacaaacattaaccaactaggaaacagct

SEQ ID NO: 16 - DNA, 203 bp, Synthetic construct
  source 1..203: mol_type = other DNA
tgcgtcgccattctgtcgcaacacgccagaatgcggcggcgatcactaactcaacaaatcaggcgatgtaaccgctttcaatctgtgagtgatttcacagtatcttaacaatgtgatagctatgattgcaccgtgcctacaagcatcgtggaggtccgtgactttcacgcatacaacaaacattaaccaaccgagaaacagct

SEQ ID NO: 17 - DNA, 310 bp, Synthetic construct
  source 1..310: mol_type = other DNA
atgcgcaaatgcggcacgccttgcagattacggtttgccacacttttcatccttctcctggtgacataatccacatcaatcgaaaatgttaataaatttgttgcgcgaatgatctaacaaacatgcatcatgtacaatcagatggaataaatggcgcgataacgctcattttatgacgaggcacacacattttaagttcgatatttctcgtttttgctcgttaacgataagtttacagcatgcctacaagcatcgtggaggtccgtgactttcacgcatacaacaaacattaaccaactaggaaacagct

SEQ ID NO: 18 - DNA, 203 bp, Synthetic construct
  source 1..203: mol_type = other DNA
tgcgtcgccattctgtcgcaacacgccagaatgcggcggcgatcactaactcaacaaatcaggcgatgtaaccgctttcaatctgtgagtgatttcacagtatcttaacaatgtgatagctatgattgcaccgtgcctacaagcatcgtggaggtccgtgactttcacgcatacaacaaacattaaccaagagcaaaacagct

SEQ ID NO: 19 - DNA, 203 bp, Synthetic construct
  source 1..203: mol_type = other DNA
tgcgtcgccattctgtcgcaacacgccagaatgcggcggcgatcactaactcaacaaatcaggcgatgtaaccgctttcaatctgtgagtgatttcacagtatcttaacaatgtgatagctatgattgcaccgtgcctacaagcatcgtggaggtccgtgactttcacgcatacaacaaacattaaccaaggaggaaacagct

SEQ ID NO: 20 - DNA, 189 bp, Synthetic construct
  source 1..189: mol_type = other DNA
gaaaacattcataaattaaatgtgaattgccgcacacattattaaataagatttacaaaatgttcaaaatgacgcatgaaatcacgtttcactttcgaattatgagcgaatatgcgcgatgcctacaagcatcgtggaggtccgtgactttcacgcatacaacaaacattaaccaaggaggaaacagct

SEQ ID NO: 21 - DNA, 239 bp, Synthetic construct
  source 1..239: mol_type = other DNA
ccatttagccatagtaaaaacatgaattgtttgatttcgcgcatattcgctcataattcgaaagtgaaacgtgatttcatgcgtcattttgaacattttgtaaatcttatttaataatgtgtgcggcaattcacatttaatttatgaatgttttcttaacatcgcggcatgcctacaagcatcgtggaggtccgtgactttcacgcatacaacaaacattaaccaaggaggaaacagct

SEQ ID NO: 22 - DNA, 300 bp, Escherichia coli
  source 1..300: mol_type = genomic DNA
gcggcacgccttgcagattacggtttgccacacttttcatccttctcctggtgacataatccacatcaatcgaaaatgttaataaatttgttgcgcgaatgatctaacaaacatgcatcatgtacaatcagatggaataaatggcgcgataacgctcattttatgacgaggcacacacattttaagttcgatatttctcgtttttgctcgttaacgataagtttacagcatgcctacaagcatcgtggaggtccgtgactttcacgcatacaacaaacattaaccaaggaggaaacagct

SEQ ID NO: 23 - DNA, 310 bp, Synthetic construct
  source 1..310: mol_type = other DNA
atgcgcaaatgcggcacgccttgcagattacggtttgccacacttttcatccttctcctggtgacataatccacatcaatcgaaaatgttaataaatttgttgcgcgaatgatctaacaaacatgcatcatgtacaatcagatggaataaatggcgcgataacgctcattttatgacgaggcacacacattttaagttcgatatttctcgtttttgctcgttaacgataagtttacagcatgcctacaagcatcgtggaggtccgtgactttcacgcatacaacaaacattaaccaactgagaaacagct

SEQ ID NO: 24 - DNA, 310 bp, Synthetic construct
  source 1..310: mol_type = other DNA
atgcgcaaatgcggcacgccttgcagattacggtttgccacacttttcatccttctcctggtgacataatccacatcaatcgaaaatgttaataaatttgttgcgcgaatgatctaacaaacatgcatcatgtacaatcagatggaataaatggcgcgataacgctcattttatgacgaggcacacacattttaagttcgatatttctcgtttttgctcgttaacgataagtttacagcatgcctacaagcatcgtggaggtccgtgactttcacgcatacaacaaacattaaccaaccgagaaacagct

SEQ ID NO: 25 - DNA, 310 bp, Synthetic construct
  source 1..310: mol_type = other DNA
atgcgcaaatgcggcacgccttgcagattacggtttgccacacttttcatccttctcctggtgacataatccacatcaatcgaaaatgttaataaatttgttgcgcgaatgatctaacaaacatgcatcatgtacaatcagatggaataaatggcgcgataacgctcattttatgacgaggcacacacattttaagttcgatatttctcgtttttgctcgttaacgataagtttacagcatgcctacaagcatcgtggaggtccgtgactttcacgcatacaacaaacattaaccaagagaaaaacagct

SEQ ID NO: 26 - DNA, 350 bp, Synthetic construct
  source 1..350: mol_type = other DNA
tgcgtcgccattctgtcgcaacacgccagaatgcggcggcgatcactaactcaacaaatcaggcgatgtaaccgctttcaatctgtgagtgatttcacagtatcttaacaatgtgatagctatgattgcaccgttttaacgttgtaacccgtatgtaacagtgaataatcacttttgccgaggtaacagcgtcataacaacaattaaagccgttttctggagcgttaccgggcatggaagaacgaattttaaaaagtgagcttcggcgttcagtaacacttcattaactctactgccccgccgagcatttatctcaagcactaccctgcataagcaaggaggaaacagct

SEQ ID NO: 27 - DNA, 310 bp, Synthetic construct
  source 1..310: mol_type = other DNA
atgcgcaaatgcggcacgccttgcagattacggtttgccacacttttcatccttctcctggtgacataatccacatcaatcgaaaatgttaataaatttgttgcgcgaatgatctaacaaacatgcatcatgtacaatcagatggaataaatggcgcgataacgctcattttatgacgaggcacacacattttaagttcgatatttctcgtttttgctcgttaacgataagtttacagcatgcctacaagcatcgtggaggtccgtgactttcacgcatacaacaaacattaaccaaaggaaaaacagct

SEQ ID NO: 28 - DNA, 300 bp, Synthetic construct
  source 1..300: mol_type = other DNA
gcggcacgccttgcagattacggtttgccacacttttcatccttctcctggtgacataatccacatcaatcgaaaatgttaataaatttgttgcgcgaatgatctaacaaacatgcatcatgtacaatcagatggaataaatggcgcgataacgctcattttatgacgaggcacacacattttaagttcgatatttctcgtttttgctcgttaacgataagtttacagcatgcctacaagcatcgtggaggtccgtgactttcacgcatacaacaaacattaaccaagagcaaaacagct

SEQ ID NO: 29 - DNA, 310 bp, Synthetic construct
  source 1..310: mol_type = other DNA
atgcgcaaatgcggcacgccttgcagattacggtttgccacacttttcatccttctcctggtgacataatccacatcaatcgaaaatgttaataaatttgttgcgcgaatgatctaacaaacatgcatcatgtacaatcagatggaataaatggcgcgataacgctcattttatgacgaggcacacacattttaagttcgatatttctcgtttttgctcgttaacgataagtttacagcatgcctacaagcatcgtggaggtccgtgactttcacgcatacaacaaacattaaccaagagctaaacagct

SEQ ID NO: 30 - DNA, 189 bp, Synthetic construct; identical to SEQ ID NO: 20
  source 1..189: mol_type = other DNA

SEQ ID NO: 31 - DNA, 107 bp, Escherichia coli
  source 1..107: mol_type = genomic DNA
tgtgagttagctcactcattaggcaccccaggctttacactttatgcttccggctcgtatgttgtgtggaattgtgagcggataacaatttcacacaggaaacagct

SEQ ID NO: 32 - DNA, 300 bp, Synthetic construct
  source 1..300: mol_type = other DNA
gcggcacgccttgcagattacggtttgccacacttttcatccttctcctggtgacataatccacatcaatcgaaaatgttaataaatttgttgcgcgaatgatctaacaaacatgcatcatgtacaatcagatggaataaatggcgcgataacgctcattttatgacgaggcacacacattttaagttcgatatttctcgtttttgctcgttaacgataagtttacagcatgcctacaagcatcgtggaggtccgtgactttcacgcatacaacaaacattaaccaagaacaaaacagct

SEQ ID NO: 33 - DNA, 300 bp, Synthetic construct
  source 1..300: mol_type = other DNA
gcggcacgccttgcagattacggtttgccacacttttcatccttctcctggtgacataatccacatcaatcgaaaatgttaataaatttgttgcgcgaatgatctaacaaacatgcatcatgtacaatcagatggaataaatggcgcgataacgctcattttatgacgaggcacacacattttaagttcgatatttctcgtttttgctcgttaacgataagtttacagcatgcctacaagcatcgtggaggtccgtgactttcacgcatacaacaaacattaaccaaattcgaaacagct

SEQ ID NO: 34 - DNA, 152 bp, Klebsiella pneumoniae
  source 1..152: mol_type = genomic DNA
ggttaacggcccactttgctggcgacatcacaattcttaaaccggtttagcaatttttattttcaccgcgttaccgacatgtttaccatatcaactaaaccggtttagcaaacattagcacactcactgatttacctttggatgtcaccaac

SEQ ID NO: 35 - DNA, 1158 bp, Escherichia coli
  source 1..1158: mol_type = genomic DNA
atgaacccagtacccgcgcaacgtgaatatttcctcgactccatccgcgcctggctgatgttgttagggataccttttcatatttctttaatctattcgagccatacatggcatgtgaatagcgccgaatcatcattgtggctgaccctttttaatgacttcatccactcgttccgcatgcaggtatttttcgttatatccggctacttttcctacatgctttttttacgctatcccttgaaaaaatggtggaaagtacgtgtcgaacgtgtaggtatcccgatgttaacagccatccccctactgacattaccgcaatttattatgctgcaatatgtcaaaggaaaagcggaaagttggcctgggctgtcattgtatgacaaatataatacgttggcctgggaattaatatcacacctgtggtttttactggtgttagtggtcatgacgacgctgtgcgtatggatatttaagcgcatcagaaataatttagaaaattctgataaaacgaataaaaaattctcgatggtaaaactatcggtgatttttttatgcctcggcatcggttatgcggtaataagaagaacgatttttattgtgtatccgcccattctgagtaatggcatgttcaattttattgtcatgcaaacgctgttttatttgccgttctttatcctcggcgcactggctttcattttccctcatcttaaagccttgtttaccacgccgtctcgtggctgtacccttgcagcagcattggcgtttgtcgcttatttactcaaccagcgctatggcagtggcgatgcctggatgtacgaaaccgagtcggtgatcaccatggtcctcggtctgtggatggtgaatgtggtcttctcctttggccaccgtttgcttaacttccagtcagcgcgggtgacttattttgttaacgcatcgctgtttatctatctggttcaccacccgttaacgctgtttttcggcgcatacattacaccgcacatcacctccaactggcttggttttctctgtggcctgatatttgtagtagggattgcgataattctgtatgaaattcatttgcgcatcccgttactgaagtttttgttctctggtaaaccggttgttaagcgtgagaacgataaagcaccagcccgttaa

SEQ ID NO: 36 - protein, 385 aa, Escherichia coli
MNPVPAQREYFLDSIRAWLMLLGIPFHISLIYSSHTWHVNSAESSLWLTLFNDFIHSFRMQVFFVISGYFSYMLFLRYPLKKWWKVRVERVGIPMLTAIPLLTLPQFIMLQYVKGKAESWPGLSLYDKYNTLAWELISHLWFLLVLVVMTTLCVWIFKRIRNNLENSDKTNKKFSMVKLSVIFLCLGIGYAVIRRTIFIVYPPILSNGMFNFIVMQTLFYLPFFILGALAFIFPHLKALFTTPSRGCTLAAALAFVAYLLNQRYGSGDAWMYETESVITMVLGLWMVNVVFSFGHRLLNFQSARVTYFVNASLFIYLVHHPLTLFFGAYITPHITSNWLGFLCGLIFVVGIAIILYEIHLRIPLLKFLFSGKPVVKRENDKAPAR